European Patent Application EP 4 502 177 A1, published February 5, 2025. Title: METHOD FOR PREPARING DNA LIBRARY AND DETECTING RETROVIRAL INTEGRATION SITE. Applicant: Nanjing Legend Biotech Co., Ltd. The sequence listing filed with the application follows.

SEQUENCE LISTING (13 sequences)

SEQ ID NO: 1 - DNA, 62 bp, synthetic construct
  source 1..62: mol_type = other DNA
acactctttccctacacgacgctcttccgatctnnnnnnnngatctgactgtctctaccagt

SEQ ID NO: 2 - DNA, 20 bp, synthetic construct
  source 1..20: mol_type = other DNA
ctggtagagacagtcagatc

SEQ ID NO: 3 - DNA, 20 bp, synthetic construct
  source 1..20: mol_type = other DNA
acactctttccctacacgac

SEQ ID NO: 4 - DNA, 20 bp, synthetic construct
  source 1..20: mol_type = other DNA
ttgccttgagtgcttcaagt

SEQ ID NO: 5 - DNA, 20 bp, synthetic construct
  source 1..20: mol_type = other DNA
cacgctttgaggtagactct

SEQ ID NO: 6 - DNA, 33 bp, synthetic construct
  source 1..33: mol_type = other DNA
acactctttccctacacgacgctcttccgatct

SEQ ID NO: 7 - DNA, 54 bp, synthetic construct
  source 1..54: mol_type = other DNA
gtgactggagttcagacgtgtgctcttccgatctagtgtgtgcccgtctgttgt

SEQ ID NO: 8 - DNA, 54 bp, synthetic construct
  source 1..54: mol_type = other DNA
gtgactggagttcagacgtgtgctcttccgatctcccgtgtataatgccacttg

SEQ ID NO: 9 - DNA, 57 bp, synthetic construct
  source 1..57: mol_type = other DNA
aatgatacggcgaccaccgagatctacacnnnnnnnnacactctttccctacacgac

SEQ ID NO: 10 - DNA, 53 bp, synthetic construct
  source 1..53: mol_type = other DNA
caagcagaagacggcatacgagatnnnnnnnngtgactggagttcagacgtgt

SEQ ID NO: 11 - DNA, 21 bp, synthetic construct
  source 1..21: mol_type = other DNA
acttgtggtctcgctgttcct

SEQ ID NO: 12 - DNA, 54 bp, synthetic construct
  source 1..54: mol_type = other DNA
gtgactggagttcagacgtgtgctcttccgatcttgggagggtctcctctgagt

SEQ ID NO: 13 - DNA, 54 bp, synthetic construct; identical to SEQ ID NO: 8
  source 1..54: mol_type = other DNA